European Patent Application EP 4 442 282 A1, published October 9, 2024. Title: Preparation of site-specific polypeptide conjugates. Applicant: POSTECH Research and Business Development Foundation. Application EP. The sequence listing filed with the application follows.

SEQUENCE LISTING (6 sequences)

SEQ ID NO: 1 - DNA, 15 bp, synthetic construct
  source 1..15: mol_type = other DNA; note = aptamer HD1
ggttggtgtggttgg

SEQ ID NO: 2 - DNA, 29 bp, synthetic construct
  source 1..29: mol_type = other DNA; note = aptamer HD2
agtccgtggtagggcaggttggggtgact

SEQ ID NO: 3 - DNA, 41 bp, synthetic construct
  source 1..41: mol_type = other DNA; note = aptamer Sgc8c
atctaactgctgcgccgccgggaaaatactgtacggttaga

SEQ ID NO: 4 - DNA, 26 bp, synthetic construct
  source 1..26: mol_type = other DNA; note = aptamer AS1411
ggtggtggtggttgtggtggtggtgg

SEQ ID NO: 5 - RNA, 23 nt, synthetic construct
  source 1..23: mol_type = other RNA; note = aptamer Apt8-2
ggaggtgctccgaaaggaactcc

SEQ ID NO: 6 - DNA, 23 bp, synthetic construct
  source 1..23: mol_type = other DNA; note = DNA complementary to Apt8-2
ggagttcctttcggagcacctcc